European Patent Application EP 4 316 526 A1, published February 7, 2024. Title: METHOD FOR CONSTRUCTION OF NUCLEIC ACID SELF-ASSEMBLY-MEDIATED ADC DRUG AND USE THEREOF. Applicant: ASSEMBLY MEDICINE, LLC. The sequence listing filed with the application follows.

SEQUENCE LISTING (7 sequences)

SEQ ID NO: 1 - protein, 165 aa, Artificial Sequence
  Anti-HER2 nanobody amino acid sequence
MSAHHHHHHWSHPQFEKGGGSGGGSGGSAWSHPQFEKENLYFQSEVQLVESGGGLVQAGGSLRLSCAASGITFSINTMGWYRQAPGKQRELVALISSIGDTYYADSVKGRFTISRDNAKNTVYLQMNSLKPEDTAVYYCKRFRTAAQGTDYWGQGTLVTVSSGSC

SEQ ID NO: 2 - protein, 163 aa, Artificial Sequence
  Anti-HSA nanobody amino acid sequence
MGSAHHHHHHWSHPQFEKGGGSGGGSGGSAWSHPQFEKENLYFQSAVQLVESGGGLVQPGNSLRLSCAASGFTFRSFGMSWVRQAPGKEPEWVSSISGSGSDTLYADSVKGRFTISRDNAKTTLYLQMNSLKPEDTAVYYCTIGGSLSRSSQGTQVTVSSGSC

SEQ ID NO: 3 - protein, 160 aa, Artificial Sequence
  Anti-PD-L1 nanobody amino acid sequence
MGSAHHHHHHWSHPQFEKGGGSGGGSGGSSAWSHPQFEKENLYFQSEVQLLESGGGEVQPGGSLRLSCAASGGIFAIKPISWYRQAPGKQREWVSTTTSSGATNYAESVKGRFTISRDNAKNTLYLQMSSLRAEDTAVYYCNVFEYWGQGTLVTVKPGSC

SEQ ID NO: 4 - DNA, 32 bp, Artificial Sequence
  L-DNA1
aggcgatcacaatccaaatgagcgtgttacgg

SEQ ID NO: 5 - DNA, 32 bp, Artificial Sequence
  L-DNA2
accgtaacacgctcaaaaccgaagtgccaatt

SEQ ID NO: 6 - DNA, 32 bp, Artificial Sequence
  L-DNA3
aaattggcacttcggaaaactatgcggctgct

SEQ ID NO: 7 - DNA, 32 bp, Artificial Sequence
  L-DNA4
aagcagccgcatagtaaaggattgtgatcgcc